European Patent Application EP 4 151 660 A1, published March 22, 2023. Title: FUSION PROTEIN FOR REVERSING TUMOR MICROENVIRONMENT AND USE THEREOF. Applicant: CHONGQING PRECISION BIOTECH COMPANY LIMITED. CHONGQING PRECISION BIOLOGICAL INDUSTRIAL TECHNOLOGY RESEARCH INSTITUTE CO., LTD. Application PCT/CN2021/095107. The sequence listing filed with the application follows.

SEQUENCE LISTING (38 sequences)

SEQ ID NO: 1 - protein, 362 aa, Artificial Sequence
  Synthesized construct
MPVPASWPHPPGPFLLLTLLLGLTEVAGEEELQMIQPEKLLLVTVGKTATLHCTVTSLLPVGPVLWFRGVGPGRELIYNQKEGHFPRVTTVSDLTKRNNMDFSIRISSITPADVGTYYCVKFRKGSPENVEFKSGPGTEMALGAKPSAPVVLGPAARTTPEHTVSFTCESHGFSPRDITLKWFKNGNELSDFQTNVDPTGQSVAYSIRSTARVVLDPWDVRSQVICEVAHVTLQGDPLRGTANLSEAIRVPPTLEVTQQPMRVGNQVNVTCQVRKFYPQSLQLTWSENGNVCQRETASTLTENKDGTYNWTSWFLVNISDQRDDVVLTCQVKHDGQLAVSKRLALEVTVHQKDQSSDATPLE

SEQ ID NO: 2 - protein, 430 aa, Artificial Sequence
  Synthesized construct
MPVPASWPHPPGPFLLLTLLLGLTEVAGEEELQMIQPEKLLLVTVGKTATLHCTVTSLLPVGPVLWFRGVGPGRELIYNQKEGHFPRVTTVSDLTKRNNMDFSIRISSITPADVGTYYCVKFRKGSPENVEFKSGPGTEMALGAKPSAPVVLGPAARTTPEHTVSFTCESHGFSPRDITLKWFKNGNELSDFQTNVDPTGQSVAYSIRSTARVVLDPWDVRSQVICEVAHVTLQGDPLRGTANLSEAIRVPPTLEVTQQPMRVGNQVNVTCQVRKFYPQSLQLTWSENGNVCQRETASTLTENKDGTYNWTSWFLVNISDQRDDVVLTCQVKHDGQLAVSKRLALEVTVHQKDQSSDATPLEFWVLVVVGGVLACYSLLVTVAFIIFWVRSKRSRGGHSDYMNMTPRRPGPTRKHYQPYAPPRDFAAYRS

SEQ ID NO: 3 - protein, 428 aa, Artificial Sequence
  Synthesized construct
MPVPASWPHPPGPFLLLTLLLGLTEVAGEEELQMIQPEKLLLVTVGKTATLHCTVTSLLPVGPVLWFRGVGPGRELIYNQKEGHFPRVTTVSDLTKRNNMDFSIRISSITPADVGTYYCVKFRKGSPENVEFKSGPGTEMALGAKPSAPVVLGPAARTTPEHTVSFTCESHGFSPRDITLKWFKNGNELSDFQTNVDPTGQSVAYSIRSTARVVLDPWDVRSQVICEVAHVTLQGDPLRGTANLSEAIRVPPTLEVTQQPMRVGNQVNVTCQVRKFYPQSLQLTWSENGNVCQRETASTLTENKDGTYNWTSWFLVNISDQRDDVVLTCQVKHDGQLAVSKRLALEVTVHQKDQSSDATPLEIYIWAPLAGTCGVLLLSLVITLYCKRGRKKLLYIFKQPFMRPVQTTQEEDGCSCRFPEEEEGGCEL

SEQ ID NO: 4 - protein, 455 aa, Artificial Sequence
  Synthesized construct
MALPVTALLLPLALLLHAARPDIQMTQSPSSLSASVGDRVTITCSTSSSVSYMHWYQQKPGKAPRLLIYSTSNLASGVPSRFSGSGSGTDFTFTISSLQPEDIATYYCHQWSSYPTFGQGTKVEIKGSTSGSGKPGSGEGSTKGQVQLQESGPGLVRPSQTLSLTCTVSGFTISSGYSWHWVRQPPGRGLEWIGYIQYSGITNYNPSLKSRVTMLVDTSKNQFSLRLSSVTAADTAVYYCAREDYDYHWYFDVWGQGSTVTVSSGAAALEKPTTTPAPRPPTPAPTIASQPLSLRPEACRPAAGGAVHTRGLDFACDEFIYIWAPLAGTCGVLLLSLVITLYCRVKFSRSADAPAYQQGQNQLYNELNLGRREEYDVLDKRRGRDPEMGGKPRRKNPQEGLYNELQKDKMAEAYSEIGMKGERRRGKGHDGLYQGLSTATKDTYDALHMQALPPR

SEQ ID NO: 5 - protein, 911 aa, Artificial Sequence
  Synthesized construct
MALPVTALLLPLALLLHAARPDIQMTQSPSSLSASVGDRVTITCSTSSSVSYMHWYQQKPGKAPRLLIYSTSNLASGVPSRFSGSGSGTDFTFTISSLQPEDIATYYCHQWSSYPTFGQGTKVEIKGSTSGSGKPGSGEGSTKGQVQLQESGPGLVRPSQTLSLTCTVSGFTISSGYSWHWVRQPPGRGLEWIGYIQYSGITNYNPSLKSRVTMLVDTSKNQFSLRLSSVTAADTAVYYCAREDYDYHWYFDVWGQGSTVTVSSGAAALEKPTTTPAPRPPTPAPTIASQPLSLRPEACRPAAGGAVHTRGLDFACDEFIYIWAPLAGTCGVLLLSLVITLYCRVKFSRSADAPAYQQGQNQLYNELNLGRREEYDVLDKRRGRDPEMGGKPRRKNPQEGLYNELQKDKMAEAYSEIGMKGERRRGKGHDGLYQGLSTATKDTYDALHMQALPPRVDGSGATNFSLLKQAGDVEENPGPSRMPVPASWPHPPGPFLLLTLLLGLTEVAGEEELQMIQPEKLLLVTVGKTATLHCTVTSLLPVGPVLWFRGVGPGRELIYNQKEGHFPRVTTVSDLTKRNNMDFSIRISSITPADVGTYYCVKFRKGSPENVEFKSGPGTEMALGAKPSAPVVLGPAARTTPEHTVSFTCESHGFSPRDITLKWFKNGNELSDFQTNVDPTGQSVAYSIRSTARVVLDPWDVRSQVICEVAHVTLQGDPLRGTANLSEAIRVPPTLEVTQQPMRVGNQVNVTCQVRKFYPQSLQLTWSENGNVCQRETASTLTENKDGTYNWTSWFLVNISDQRDDVVLTCQVKHDGQLAVSKRLALEVTVHQKDQSSDATPLEFWVLVVVGGVLACYSLLVTVAFIIFWVRSKRSRGGHSDYMNMTPRRPGPTRKHYQPYAPPRDFAAYRS

SEQ ID NO: 6 - protein, 907 aa, Artificial Sequence
  Synthesized construct
MALPVTALLLPLALLLHAARPDIQMTQSPSSLSASVGDRVTITCSTSSSVSYMHWYQQKPGKAPRLLIYSTSNLASGVPSRFSGSGSGTDFTFTISSLQPEDIATYYCHQWSSYPTFGQGTKVEIKGSTSGSGKPGSGEGSTKGQVQLQESGPGLVRPSQTLSLTCTVSGFTISSGYSWHWVRQPPGRGLEWIGYIQYSGITNYNPSLKSRVTMLVDTSKNQFSLRLSSVTAADTAVYYCAREDYDYHWYFDVWGQGSTVTVSSGAAALEKPTTTPAPRPPTPAPTIASQPLSLRPEACRPAAGGAVHTRGLDFACDEFIYIWAPLAGTCGVLLLSLVITLYCRVKFSRSADAPAYQQGQNQLYNELNLGRREEYDVLDKRRGRDPEMGGKPRRKNPQEGLYNELQKDKMAEAYSEIGMKGERRRGKGHDGLYQGLSTATKDTYDALHMQALPPRVDGSGATNFSLLKQAGDVEENPGPMPVPASWPHPPGPFLLLTLLLGLTEVAGEEELQMIQPEKLLLVTVGKTATLHCTVTSLLPVGPVLWFRGVGPGRELIYNQKEGHFPRVTTVSDLTKRNNMDFSIRISSITPADVGTYYCVKFRKGSPENVEFKSGPGTEMALGAKPSAPVVLGPAARTTPEHTVSFTCESHGFSPRDITLKWFKNGNELSDFQTNVDPTGQSVAYSIRSTARVVLDPWDVRSQVICEVAHVTLQGDPLRGTANLSEAIRVPPTLEVTQQPMRVGNQVNVTCQVRKFYPQSLQLTWSENGNVCQRETASTLTENKDGTYNWTSWFLVNISDQRDDVVLTCQVKHDGQLAVSKRLALEVTVHQKDQSSDATPLEIYIWAPLAGTCGVLLLSLVITLYCKRGRKKLLYIFKQPFMRPVQTTQEEDGCSCRFPEEEEGGCEL

SEQ ID NO: 7 - protein, 27 aa, Artificial Sequence
  Synthesized construct
FWVLVVVGGVLACYSLLVTVAFIIFWV

SEQ ID NO: 8 - protein, 24 aa, Artificial Sequence
  Synthesized construct
IYIWAPLAGTCGVLLLSLVITLYC

SEQ ID NO: 9 - protein, 41 aa, Artificial Sequence
  Synthesized construct
RSKRSRLLHSDYMNMTPRRPGPTRKHYQPYAPPRDFAAYRS

SEQ ID NO: 10 - protein, 44 aa, Artificial Sequence
  Synthesized construct
VKRGRKKLLYIFKQPFMRPVQTTQEEDGCSCRFPEEEEGGCELR

SEQ ID NO: 11 - protein, 111 aa, Artificial Sequence
  Synthesized construct
VKFSRSADAPAYQQGQNQLYNELNLGRREEYDVLDKRRGRDPEMGGKPRRKNPQEGLYNELQKDKMAEAYSEIGMKGERRRGKGHDGLYQGLSTATKDTYDALHMQALPPR

SEQ ID NO: 12 - DNA, 1086 bp, Artificial Sequence
  Synthesized construct
atgcctgtcccagcctcctggccccatcctcctggtcctttcctgcttctgactctactgctgggacttacagaagtggcaggtgaggaggagctacagatgattcagcctgagaagctcctgttggtcacagttggaaagacagccactctgcactgcactgtgacctccctgcttcccgtgggacccgtcctgtggttcagaggagttggaccaggccgggaattaatctacaatcaaaaagaaggccacttccccagggtaacaacagtttcagacctcacaaagagaaacaacatggacttttccatccgcatcagtagcatcaccccagcagatgtcggcacatactactgtgtgaagtttcgaaaagggagccctgagaacgtggagtttaagtctggaccaggcactgagatggctttgggtgccaaaccctctgcccccgtggtattgggccctgcggcgaggaccacacctgagcatacagtgagtttcacctgtgagtcccatggcttctctcccagagacatcaccctgaaatggttcaaaaatgggaatgagctctcagacttccagaccaacgtggaccccacaggacagagtgtggcctacagcatccgcagcacagccagggtggtactggacccctgggacgttcgctctcaggtcatctgcgaggtggcccatgtcaccttgcagggggaccctcttcgtgggactgccaacttgtctgaggccatccgagttccacccaccttggaggttactcaacagcccatgagggtggggaaccaggtaaacgtcacctgccaggtgaggaagttctacccccagagcctacagctgacctggtcggagaatggaaacgtgtgccagagagaaacagcctcgacccttacagagaacaaggatggtacctacaactggacaagctggttcctggtgaacatatctgaccaaagggatgatgtggtcctcacctgccaggtgaagcatgatgggcagctggcggtcagcaaacgccttgccctagaggtcacagtccaccagaaggaccagagctcagatgctacccctctcgag

SEQ ID NO: 13 - DNA, 1290 bp, Artificial Sequence
  Synthesized construct
atgcctgtcccagcctcctggccccatcctcctggtcctttcctgcttctgactctactgctgggacttacagaagtggcaggtgaggaggagctacagatgattcagcctgagaagctcctgttggtcacagttggaaagacagccactctgcactgcactgtgacctccctgcttcccgtgggacccgtcctgtggttcagaggagttggaccaggccgggaattaatctacaatcaaaaagaaggccacttccccagggtaacaacagtttcagacctcacaaagagaaacaacatggacttttccatccgcatcagtagcatcaccccagcagatgtcggcacatactactgtgtgaagtttcgaaaagggagccctgagaacgtggagtttaagtctggaccaggcactgagatggctttgggtgccaaaccctctgcccccgtggtattgggccctgcggcgaggaccacacctgagcatacagtgagtttcacctgtgagtcccatggcttctctcccagagacatcaccctgaaatggttcaaaaatgggaatgagctctcagacttccagaccaacgtggaccccacaggacagagtgtggcctacagcatccgcagcacagccagggtggtactggacccctgggacgttcgctctcaggtcatctgcgaggtggcccatgtcaccttgcagggggaccctcttcgtgggactgccaacttgtctgaggccatccgagttccacccaccttggaggttactcaacagcccatgagggtggggaaccaggtaaacgtcacctgccaggtgaggaagttctacccccagagcctacagctgacctggtcggagaatggaaacgtgtgccagagagaaacagcctcgacccttacagagaacaaggatggtacctacaactggacaagctggttcctggtgaacatatctgaccaaagggatgatgtggtcctcacctgccaggtgaagcatgatgggcagctggcggtcagcaaacgccttgccctagaggtcacagtccaccagaaggaccagagctcagatgctacccctctcgagttctgggtgctggtcgtggtgggtggcgtgctggcctgctacagcctgctggtgacagtggccttcatcatcttttgggtgaggagcaagcggagcagaggcggccacagcgactacatgaacatgactccccgccgccccgggcccacccgcaagcattaccagccctatgccccaccacgcgacttcgcagcctatcgctcc

SEQ ID NO: 14 - DNA, 1284 bp, Artificial Sequence
  Synthesized construct
atgcctgtcccagcctcctggccccatcctcctggtcctttcctgcttctgactctactgctgggacttacagaagtggcaggtgaggaggagctacagatgattcagcctgagaagctcctgttggtcacagttggaaagacagccactctgcactgcactgtgacctccctgcttcccgtgggacccgtcctgtggttcagaggagttggaccaggccgggaattaatctacaatcaaaaagaaggccacttccccagggtaacaacagtttcagacctcacaaagagaaacaacatggacttttccatccgcatcagtagcatcaccccagcagatgtcggcacatactactgtgtgaagtttcgaaaagggagccctgagaacgtggagtttaagtctggaccaggcactgagatggctttgggtgccaaaccctctgcccccgtggtattgggccctgcggcgaggaccacacctgagcatacagtgagtttcacctgtgagtcccatggcttctctcccagagacatcaccctgaaatggttcaaaaatgggaatgagctctcagacttccagaccaacgtggaccccacaggacagagtgtggcctacagcatccgcagcacagccagggtggtactggacccctgggacgttcgctctcaggtcatctgcgaggtggcccatgtcaccttgcagggggaccctcttcgtgggactgccaacttgtctgaggccatccgagttccacccaccttggaggttactcaacagcccatgagggtggggaaccaggtaaacgtcacctgccaggtgaggaagttctacccccagagcctacagctgacctggtcggagaatggaaacgtgtgccagagagaaacagcctcgacccttacagagaacaaggatggtacctacaactggacaagctggttcctggtgaacatatctgaccaaagggatgatgtggtcctcacctgccaggtgaagcatgatgggcagctggcggtcagcaaacgccttgccctagaggtcacagtccaccagaaggaccagagctcagatgctacccctctcgagatctacatctgggcgcccttggccgggacttgtggggtccttctcctgtcactggttatcaccctttactgcaaacggggcagaaagaaactcctgtatatattcaaacaaccatttatgagaccagtacaaactactcaagaggaagatggctgtagctgccgatttccagaagaagaagaaggaggatgtgaactg

SEQ ID NO: 15 - DNA, 1365 bp, Artificial Sequence
  Synthesized construct
atggccttaccagtgaccgccttgctcctgccgctggccttgctgctccacgccgccaggccggacatccagatgacccagagcccaagcagcctgagcgccagcgtgggtgacagagtgaccatcacctgtagtaccagttcgagtgtaagttacatgcactggtaccagcagaagccaggtaaggctccaaggctgctgatctacagcacatccaacctggcttctggtgtgccaagcagattcagcggtagcggtagcggtaccgacttcaccttcaccatcagcagcctccagccagaggacatcgccacctactactgccatcagtggagtagttatcccacgttcggccaagggaccaaggtggaaatcaaaggatccacttccggttcaggaaagcccgggagtggtgaaggtagcactaaaggccaggtccagctgcaggagagcggtccaggtcttgtgagacctagccagaccctgagcctgacctgcaccgtgtctggcttcaccatcagcagtggttatagctggcactgggtgagacagccacctggacgaggtcttgagtggattggatacatacagtacagtggtatcactaactacaacccctctctcaaaagtagagtgacaatgctggtagacaccagcaagaaccagttcagcctgagactcagcagcgtgacagccgccgacaccgcggtctattattgtgcaagagaagactatgattaccactggtacttcgatgtctggggtcaaggcagcacggtcaccgtctcctcaggtgcggccgccctcgagaagcccaccacgacgccagcgccgcgaccaccaacaccggcgcccaccatcgcgtcgcagcccctgtccctgcgcccagaggcgtgccggccagcggcggggggcgcagtgcacacgagggggctggacttcgcctgcgacgaattcatctacatctgggcacccctggccggaacttgtggagtgctgctgctgtctctggtcattaccctgtattgtagagtgaagttcagcaggagcgcagacgcccccgcgtaccagcagggccagaaccagctctataacgagctcaatctaggacgaagagaggagtacgatgttttggacaagagacgtggccgggaccctgagatggggggaaagccgagaaggaagaaccctcaggaaggcctgtacaatgaactgcagaaagataagatggcggaggcctacagtgagattgggatgaaaggcgagcgccggaggggcaaggggcacgatggcctttaccagggtctcagtacagccaccaaggacacctacgacgcccttcacatgcaggccctgccccctcgc

SEQ ID NO: 16 - DNA, 2736 bp, Artificial Sequence
  Synthesized construct
atggccttaccagtgaccgccttgctcctgccgctggccttgctgctccacgccgccaggccggacatccagatgacccagagcccaagcagcctgagcgccagcgtgggtgacagagtgaccatcacctgtagtaccagttcgagtgtaagttacatgcactggtaccagcagaagccaggtaaggctccaaggctgctgatctacagcacatccaacctggcttctggtgtgccaagcagattcagcggtagcggtagcggtaccgacttcaccttcaccatcagcagcctccagccagaggacatcgccacctactactgccatcagtggagtagttatcccacgttcggccaagggaccaaggtggaaatcaaaggatccacttccggttcaggaaagcccgggagtggtgaaggtagcactaaaggccaggtccagctgcaggagagcggtccaggtcttgtgagacctagccagaccctgagcctgacctgcaccgtgtctggcttcaccatcagcagtggttatagctggcactgggtgagacagccacctggacgaggtcttgagtggattggatacatacagtacagtggtatcactaactacaacccctctctcaaaagtagagtgacaatgctggtagacaccagcaagaaccagttcagcctgagactcagcagcgtgacagccgccgacaccgcggtctattattgtgcaagagaagactatgattaccactggtacttcgatgtctggggtcaaggcagcacggtcaccgtctcctcaggtgcggccgccctcgagaagcccaccacgacgccagcgccgcgaccaccaacaccggcgcccaccatcgcgtcgcagcccctgtccctgcgcccagaggcgtgccggccagcggcggggggcgcagtgcacacgagggggctggacttcgcctgcgacgaattcatctacatctgggcacccctggccggaacttgtggagtgctgctgctgtctctggtcattaccctgtattgtagagtgaagttcagcaggagcgcagacgcccccgcgtaccagcagggccagaaccagctctataacgagctcaatctaggacgaagagaggagtacgatgttttggacaagagacgtggccgggaccctgagatggggggaaagccgagaaggaagaaccctcaggaaggcctgtacaatgaactgcagaaagataagatggcggaggcctacagtgagattgggatgaaaggcgagcgccggaggggcaaggggcacgatggcctttaccagggtctcagtacagccaccaaggacacctacgacgcccttcacatgcaggccctgccccctcgcgtcgacggaagcggagctactaacttcagcctgctgaagcaggctggagacgtggaggagaaccctggaccttctagaatgcctgtcccagcctcctggccccatcctcctggtcctttcctgcttctgactctactgctgggacttacagaagtggcaggtgaggaggagctacagatgattcagcctgagaagctcctgttggtcacagttggaaagacagccactctgcactgcactgtgacctccctgcttcccgtgggacccgtcctgtggttcagaggagttggaccaggccgggaattaatctacaatcaaaaagaaggccacttccccagggtaacaacagtttcagacctcacaaagagaaacaacatggacttttccatccgcatcagtagcatcaccccagcagatgtcggcacatactactgtgtgaagtttcgaaaagggagccctgagaacgtggagtttaagtctggaccaggcactgagatggctttgggtgccaaaccctctgcccccgtggtattgggccctgcggcgaggaccacacctgagcatacagtgagtttcacctgtgagtcccatggcttctctcccagagacatcaccctgaaatggttcaaaaatgggaatgagctctcagacttccagaccaacgtggaccccacaggacagagtgtggcctacagcatccgcagcacagccagggtggtactggacccctgggacgttcgctctcaggtcatctgcgaggtggcccatgtcaccttgcagggggaccctcttcgtgggactgccaacttgtctgaggccatccgagttccacccaccttggaggttactcaacagcccatgagggtggggaaccaggtaaacgtcacctgccaggtgaggaagttctacccccagagcctacagctgacctggtcggagaatggaaacgtgtgccagagagaaacagcctcgacccttacagagaacaaggatggtacctacaactggacaagctggttcctggtgaacatatctgaccaaagggatgatgtggtcctcacctgccaggtgaagcatgatgggcagctggcggtcagcaaacgccttgccctagaggtcacagtccaccagaaggaccagagctcagatgctacccctctcgagttctgggtgctggtcgtggtgggtggcgtgctggcctgctacagcctgctggtgacagtggccttcatcatcttttgggtgaggagcaagcggagcagaggcggccacagcgactacatgaacatgactccccgccgccccgggcccacccgcaagcattaccagccctatgccccaccacgcgacttcgcagcctatcgctcctaa

SEQ ID NO: 17 - DNA, 2724 bp, Artificial Sequence
  Synthesized construct
atggccttaccagtgaccgccttgctcctgccgctggccttgctgctccacgccgccaggccggacatccagatgacccagagcccaagcagcctgagcgccagcgtgggtgacagagtgaccatcacctgtagtaccagttcgagtgtaagttacatgcactggtaccagcagaagccaggtaaggctccaaggctgctgatctacagcacatccaacctggcttctggtgtgccaagcagattcagcggtagcggtagcggtaccgacttcaccttcaccatcagcagcctccagccagaggacatcgccacctactactgccatcagtggagtagttatcccacgttcggccaagggaccaaggtggaaatcaaaggatccacttccggttcaggaaagcccgggagtggtgaaggtagcactaaaggccaggtccagctgcaggagagcggtccaggtcttgtgagacctagccagaccctgagcctgacctgcaccgtgtctggcttcaccatcagcagtggttatagctggcactgggtgagacagccacctggacgaggtcttgagtggattggatacatacagtacagtggtatcactaactacaacccctctctcaaaagtagagtgacaatgctggtagacaccagcaagaaccagttcagcctgagactcagcagcgtgacagccgccgacaccgcggtctattattgtgcaagagaagactatgattaccactggtacttcgatgtctggggtcaaggcagcacggtcaccgtctcctcaggtgcggccgccctcgagaagcccaccacgacgccagcgccgcgaccaccaacaccggcgcccaccatcgcgtcgcagcccctgtccctgcgcccagaggcgtgccggccagcggcggggggcgcagtgcacacgagggggctggacttcgcctgcgacgaattcatctacatctgggcacccctggccggaacttgtggagtgctgctgctgtctctggtcattaccctgtattgtagagtgaagttcagcaggagcgcagacgcccccgcgtaccagcagggccagaaccagctctataacgagctcaatctaggacgaagagaggagtacgatgttttggacaagagacgtggccgggaccctgagatggggggaaagccgagaaggaagaaccctcaggaaggcctgtacaatgaactgcagaaagataagatggcggaggcctacagtgagattgggatgaaaggcgagcgccggaggggcaaggggcacgatggcctttaccagggtctcagtacagccaccaaggacacctacgacgcccttcacatgcaggccctgccccctcgcgtcgacggaagcggagctactaacttcagcctgctgaagcaggctggagacgtggaggagaaccctggacctatgcctgtcccagcctcctggccccatcctcctggtcctttcctgcttctgactctactgctgggacttacagaagtggcaggtgaggaggagctacagatgattcagcctgagaagctcctgttggtcacagttggaaagacagccactctgcactgcactgtgacctccctgcttcccgtgggacccgtcctgtggttcagaggagttggaccaggccgggaattaatctacaatcaaaaagaaggccacttccccagggtaacaacagtttcagacctcacaaagagaaacaacatggacttttccatccgcatcagtagcatcaccccagcagatgtcggcacatactactgtgtgaagtttcgaaaagggagccctgagaacgtggagtttaagtctggaccaggcactgagatggctttgggtgccaaaccctctgcccccgtggtattgggccctgcggcgaggaccacacctgagcatacagtgagtttcacctgtgagtcccatggcttctctcccagagacatcaccctgaaatggttcaaaaatgggaatgagctctcagacttccagaccaacgtggaccccacaggacagagtgtggcctacagcatccgcagcacagccagggtggtactggacccctgggacgttcgctctcaggtcatctgcgaggtggcccatgtcaccttgcagggggaccctcttcgtgggactgccaacttgtctgaggccatccgagttccacccaccttggaggttactcaacagcccatgagggtggggaaccaggtaaacgtcacctgccaggtgaggaagttctacccccagagcctacagctgacctggtcggagaatggaaacgtgtgccagagagaaacagcctcgacccttacagagaacaaggatggtacctacaactggacaagctggttcctggtgaacatatctgaccaaagggatgatgtggtcctcacctgccaggtgaagcatgatgggcagctggcggtcagcaaacgccttgccctagaggtcacagtccaccagaaggaccagagctcagatgctacccctctcgagatctacatctgggcgcccttggccgggacttgtggggtccttctcctgtcactggttatcaccctttactgcaaacggggcagaaagaaactcctgtatatattcaaacaaccatttatgagaccagtacaaactactcaagaggaagatggctgtagctgccgatttccagaagaagaagaaggaggatgtgaactgtaa

SEQ ID NO: 18 - DNA, 81 bp, Artificial Sequence
  Synthesized construct
ttctgggtgctggtcgtggtgggtggcgtgctggcctgctacagcctgctggtgacagtggccttcatcatcttttgggtg

SEQ ID NO: 19 - DNA, 72 bp, Artificial Sequence
  Synthesized construct
atctacatctgggcgcccttggccgggacttgtggggtccttctcctgtcactggttatcaccctttactgc

SEQ ID NO: 20 - DNA, 123 bp, Artificial Sequence
  Synthesized construct
aggagcaagcggagcagaggcggccacagcgactacatgaacatgaccccccggaggcctggccccacccggaagcactaccagccctacgcccctcccagggacttcgccgcctaccggagc

SEQ ID NO: 21 - DNA, 126 bp, Artificial Sequence
  Synthesized construct
aaacggggcagaaagaaactcctgtatatattcaaacaaccatttatgagaccagtacaaactactcaagaggaagatggctgtagctgccgatttccagaagaagaagaaggaggatgtgaactg

SEQ ID NO: 22 - DNA, 336 bp, Artificial Sequence
  Synthesized construct
agagtgaagttcagcaggagcgcagacgcccccgcgtacaagcagggccagaaccagctctataacgagctcaatctaggacgaagagaggagtacgatgttttggacaagagacgtggccgggaccctgagatggggggaaagccgagaaggaagaaccctcaggaaggcctgtacaatgaactgcagaaagataagatggcggaggcctacagtgagattgggatgaaaggcgagcgccggaggggcaaggggcacgatggcctttaccagggtctcagtacagccaccaaggacacctacgacgcccttcacatgcaggccctgccccctcgc

SEQ ID NO: 23 - protein, 496 aa, Artificial Sequence
  Synthesized construct
MALPVTALLLPLALLLHAARPDIQMTQSPSSLSASVGDRVTITCSTSSSVSYMHWYQQKPGKAPRLLIYSTSNLASGVPSRFSGSGSGTDFTFTISSLQPEDIATYYCHQWSSYPTFGQGTKVEIKGSTSGSGKPGSGEGSTKGQVQLQESGPGLVRPSQTLSLTCTVSGFTISSGYSWHWVRQPPGRGLEWIGYIQYSGITNYNPSLKSRVTMLVDTSKNQFSLRLSSVTAADTAVYYCAREDYDYHWYFDVWGQGSTVTVSSGAAALEKPTTTPAPRPPTPAPTIASQPLSLRPEACRPAAGGAVHTRGLDFACDIYIWAPLAGTCGVLLLSLVITLYCVKRGRKKLLYIFKQPFMRPVQTTQEEDGCSCRFPEEEEGGCELRVKFSRSADAPAYQQGQNQLYNELNLGRREEYDVLDKRRGRDPEMGGKPRRKNPQEGLYNELQKDKMAEAYSEIGMKGERRRGKGHDGLYQGLSTATKDTYDALHMQALPPR

SEQ ID NO: 24 - protein, 47 aa, Artificial Sequence
  Synthesized construct
KPTTTPAPRPPTPAPTIASQPLSLRPEACRPAAGGAVHTRGLDFACD

SEQ ID NO: 25 - protein, 264 aa, Artificial Sequence
  Synthesized construct
MALPVTALLLPLALLLHAARPDIQMTQSPSSLSASVGDRVTITCSTSSSVSYMHWYQQKPGKAPRLLIYSTSNLASGVPSRFSGSGSGTDFTFTISSLQPEDIATYYCHQWSSYPTFGQGTKVEIKGSTSGSGKPGSGEGSTKGQVQLQESGPGLVRPSQTLSLTCTVSGFTISSGYSWHWVRQPPGRGLEWIGYIQYSGITNYNPSLKSRVTMLVDTSKNQFSLRLSSVTAADTAVYYCAREDYDYHWYFDVWGQGSTVTVSS

SEQ ID NO: 26 - protein, 493 aa, Artificial Sequence
  Synthesized construct
MALPVTALLLPLALLLHAARPDIQMTQSPSSLSASVGDRVTITCSTSSSVSYMHWYQQKPGKAPRLLIYSTSNLASGVPSRFSGSGSGTDFTFTISSLQPEDIATYYCHQWSSYPTFGQGTKVEIKGSTSGSGKPGSGEGSTKGQVQLQESGPGLVRPSQTLSLTCTVSGFTISSGYSWHWVRQPPGRGLEWIGYIQYSGITNYNPSLKSRVTMLVDTSKNQFSLRLSSVTAADTAVYYCAREDYDYHWYFDVWGQGSTVTVSSGAAALETTTPAPRPPTPAPTIASQPLSLRPEACRPAAGGAVHTRGLDFACDIYIWAPLAGTCGVLLLSLVITLYCKRGRKKLLYIFKQPFMRPVQTTQEEDGCSCRFPEEEEGGCELRVKFSRSADAPAYKQGQNQLYNELNLGRREEYDVLDKRRGRDPEMGGKPRRKNPQEGLYNELQKDKMAEAYSEIGMKGERRRGKGHDGLYQGLSTATKDTYDALHMQALPPR

SEQ ID NO: 27 - protein, 470 aa, Artificial Sequence
  Synthesized construct
DIQMTQSPSSLSASVGDRVTITCRASQDISKYLNWYQQKPGKAPRLLIYHTSRLHSGVPSRFSGSGSGTDYTLTISSLQPEDFATYYCQQGNTLPYTFGGGTRLEIKGSTSGSGKPGSGEGSTKGQVQLQESGPGLVKPSQTLSLTCTVSGVSLPDYGVSWIRQPPGKALEWLGVIWGSETTYYNSSLKTRLTISKDNSKNQVVLTMTNMDPVDTATYYCAKHYYYGGSYAMDYWGQGSSVTVSSLETTTPAPRPPTPAPTIASQPLSLRPEACRPAAGGAVHTRGLDFACDIYIWAPLAGTCGVLLLSLVITLYCKRGRKKLLYIFKQPFMRPVQTTQEEDGCSCRFPEEEEGGCELRVKFSRSADAPAYKQGQNQLYNELNLGRREEYDVLDKRRGRDPEMGGKPRRKNPQEGLYNELQKDKMAEAYSEIGMKGERRRGKGHDGLYQGLSTATKDTYDALHMQALPPR

SEQ ID NO: 28 - protein, 696 aa, Artificial Sequence
  Synthesized construct
DIQDIQLTQSPSSLSASVGDRVTITCSASSSVRFIHWYQQKPGKAPKRLIYDTSKLASGVPSRFSGSGSGTDFTLTISSLQPEDFATYYCQQWSSSPFTFGQGTKVEIKGSTSGSGKPGSGEGSTKGSEVQLVESGGGLVQPGGSLRLSCAASGFNIKDYYIHWVRQAPGKGLEWVAWIDPENGDTEFVPKFQGRATISADTSKNTAYLQMNSLRAEDTAVYYCKTGGFWGQGTLVTVSSLEESKYGPPCPPCPAPEFLGGPSVFLFPPKPKDTLMISRTPEVTCVVVDVSQEDPEVQFNWYVDGVEVHNAKTKPREEQFNSTYRVVSVLTVLHQDWLNGKEYKCKVSNKGLPSSIEKTISKAKGQPREPQVYTLPPSQEEMTKNQVSLTCLVKGFYPSDIAVEWESNGQPENNYKTTPPVLDSDGSFFLYSRLTVDKSRWQEGNVFSCSVMHEALHNHYTQKSLSLSLGKEFFWVLVVVGGVLACYSLLVTVAFIIFWVRSKRSRGGHSDYMNMTPRRPGPTRKHYQPYAPPRDFAAYRSVKRGRKKLLYIFKQPFMRPVQTTQEEDGCSCRFPEEEEGGCELRVKFSRSADAPAYQQGQNQLYNELNLGRREEYDVLDKRRGRDPEMGGKPRRKNPQEGLYNELQKDKMAEAYSEIGMKGERRRGKGHDGLYQGLSTATKDTYDALHMQALPPR

SEQ ID NO: 29 - protein, 503 aa, Artificial Sequence
  Synthesized construct
DIQDIQLTQSPSSLSASVGDRVTITCSASSSVRFIHWYQQKPGKAPKRLIYDTSKLASGVPSRFSGSGSGTDFTLTISSLQPEDFATYYCQQWSSSPFTFGQGTKVEIKGSTSGSGKPGSGEGSTKGSEVQLVESGGGLVQPGGSLRLSCAASGFNIKDYYIHWVRQAPGKGLEWVAWIDPENGDTEFVPKFQGRATISADTSKNTAYLQMNSLRAEDTAVYYCKTGGFWGQGTLVTVSSLEAPPRASALPAPPTGSALPDPQTASALPDPPAASALPEFFWVLVVVGGVLACYSLLVTVAFIIFWVRSKRSRGGHSDYMNMTPRRPGPTRKHYQPYAPPRDFAAYRSVKRGRKKLLYIFKQPFMRPVQTTQEEDGCSCRFPEEEEGGCELRVKFSRSADAPAYQQGQNQLYNELNLGRREEYDVLDKRRGRDPEMGGKPRRKNPQEGLYNELQKDKMAEAYSEIGMKGERRRGKGHDGLYQGLSTATKDTYDALHMQALPPR

SEQ ID NO: 30 - DNA, 277 bp, Artificial Sequence
  Synthesized construct
atcccacagtgcatacgtgggctccaacaggtcctcttgtcgagccacagtgcatacgtgggctccaacaggtcctcttgtcgagccacagtgcatacgtgggctccaacaggtcctcttgtcgagccacagtgcatacgtgggctccaacaggtcctcttgtcgagccacagtgcatacgtgggctccaacaggtcctcttgtcgagatctggtaggcgtgtacggtgggaggtctatataagcagagctcgtttagtgaaccgtcagatcactag

SEQ ID NO: 31 - DNA, 2778 bp, Artificial Sequence
  Synthesized construct
gacatccagatgacccagagcccaagcagcctgagcgccagcgtgggtgacagagtgaccatcacctgtagtaccagttcgagtgtaagttacatgcactggtaccagcagaagccaggtaaggctccaaggctgctgatctacagcacatccaacctggcttctggtgtgccaagcagattcagcggtagcggtagcggtaccgacttcaccttcaccatcagcagcctccagccagaggacatcgccacctactactgccatcagtggagtagttatcccacgttcggccaagggaccaaggtggaaatcaaaggatccacttccggttcaggaaagcccgggagtggtgaaggtagcactaaaggccaggtccagctgcaggagagcggtccaggtcttgtgagacctagccagaccctgagcctgacctgcaccgtgtctggcttcaccatcagcagtggttatagctggcactgggtgagacagccacctggacgaggtcttgagtggattggatacatacagtacagtggtatcactaactacaacccctctctcaaaagtagagtgacaatgctggtagacaccagcaagaaccagttcagcctgagactcagcagcgtgacagccgccgacaccgcggtctattattgtgcaagagaagactatgattaccactggtacttcgatgtctggggtcaaggcagcacggtcaccgtctcctcaggtgcggccgccctcgagaccacgacgccagcgccgcgaccaccaacaccggcgcccaccatcgcgtcgcagcccctgtccctgcgcccagaggcgtgccggccagcggcggggggcgcagtgcacacgagggggctggacttcgcctgtgatatctacatctgggcgcccttggccgggacttgtggggtccttctcctgtcactggttatcaccctttactgcaaacggggcagaaagaaactcctgtatatattcaaacaaccatttatgagaccagtacaaactactcaagaggaagatggctgtagctgccgatttccagaagaagaagaaggaggatgtgaactgagagtgaagttcagcaggagcgcagacgcccccgcgtacaagcagggccagaaccagctctataacgagctcaatctaggacgaagagaggagtacgatgttttggacaagagacgtggccgggaccctgagatggggggaaagccgagaaggaagaaccctcaggaaggcctgtacaatgaactgcagaaagataagatggcggaggcctacagtgagattgggatgaaaggcgagcgccggaggggcaaggggcacgatggcctttaccagggtctcagtacagccaccaaggacacctacgacgcccttcacatgcaggccctgccccctcgcgtcgacggaagcggagctactaacttcagcctgctgaagcaggctggagacgtggaggagaaccctggacctatgcctgtcccagcctcctggccccatcctcctggtcctttcctgcttctgactctactgctgggacttacagaagtggcaggtgaggaggagctacagatgattcagcctgagaagctcctgttggtcacagttggaaagacagccactctgcactgcactgtgacctccctgcttcccgtgggacccgtcctgtggttcagaggagttggaccaggccgggaattaatctacaatcaaaaagaaggccacttccccagggtaacaacagtttcagacctcacaaagagaaacaacatggacttttccatccgcatcagtagcatcaccccagcagatgtcggcacatactactgtgtgaagtttcgaaaagggagccctgagaacgtggagtttaagtctggaccaggcactgagatggctttgggtgccaaaccctctgcccccgtggtattgggccctgcggcgaggaccacacctgagcatacagtgagtttcacctgtgagtcccatggcttctctcccagagacatcaccctgaaatggttcaaaaatgggaatgagctctcagacttccagaccaacgtggaccccacaggacagagtgtggcctacagcatccgcagcacagccagggtggtactggacccctgggacgttcgctctcaggtcatctgcgaggtggcccatgtcaccttgcagggggaccctcttcgtgggactgccaacttgtctgaggccatccgagttccacccaccttggaggttactcaacagcccatgagggtggggaaccaggtaaacgtcacctgccaggtgaggaagttctacccccagagcctacagctgacctggtcggagaatggaaacgtgtgccagagagaaacagcctcgacccttacagagaacaaggatggtacctacaactggacaagctggttcctggtgaacatatctgaccaaagggatgatgtggtcctcacctgccaggtgaagcatgatgggcagctggcggtcagcaaacgccttgccctagaggtcacagtccaccagaaggaccagagctcagatgctacccctcttgagttctgggtgctggtcgtggtgggtggcgtgctggcctgctacagcctgctggtgacagtggccttcatcatcttttgggtgaggagcaagcggagcagaggcggccacagcgactacatgaacatgactccccgccgccccgggcccacccgcaagcattaccagccctatgccccaccacgcgacttcgcagcctatcgctcc

SEQ ID NO: 32 - DNA, 1473 bp, Artificial Sequence
  Synthesized construct
atggctctgccagtgacagctctgctgctgcctctggctctgctgctgcacgcagctagacccgacatccagatgacccagagcccttcttctctgagcgccagcgtgggagacagagtgaccatcacttgcagggccagccaggacatcagcaagtacctgaattggtaccagcagaagccaggcaaggcccctagactgctgatctaccacacaagcagactgcacagcggagtgcctagcagattcagcggcagcggaagcggaaccgactacaccctgaccatcagcagcctgcagccagaggacttcgccacctactactgccagcagggcaacacactgccttacaccttcggcggaggcacaagactggagatcaagggcagcacaagcggaagcggcaaaccaggaagcggagaaggaagcaccaagggacaggtgcagctgcaggaaagcggaccaggactggtgaagccttctcagaccctgagcctgacttgcaccgtgtcaggagtgtccctgccagattacggcgtgtcttggatcagacagcccccaggaaaggccctggagtggctgggagtgatttggggaagcgagaccacctactacaacagcagcctgaagacccggctgaccatcagcaaggacaacagcaagaaccaggtggtgctgaccatgaccaacatggaccccgtggacaccgccacctactattgcgccaagcactactactacggcggaagctacgccatggactattggggccagggaagcagcgtgaccgtgtctagcctcgagaccacgacgccagcgccgcgaccaccaacaccggcgcccaccatcgcgtcgcagcccctgtccctgcgcccagaggcgtgccggccagcggcggggggcgcagtgcacacgagggggctggacttcgcctgtgatatctacatctgggcgcccttggccgggacttgtggggtccttctcctgtcactggttatcaccctttactgcaaacggggcagaaagaaactcctgtatatattcaaacaaccatttatgagaccagtacaaactactcaagaggaagatggctgtagctgccgatttccagaagaagaagaaggaggatgtgaactgagagtgaagttcagcaggagcgcagacgcccccgcgtacaagcagggccagaaccagctctataacgagctcaatctaggacgaagagaggagtacgatgttttggacaagagacgtggccgggaccctgagatggggggaaagccgagaaggaagaaccctcaggaaggcctgtacaatgaactgcagaaagataagatggcggaggcctacagtgagattgggatgaaaggcgagcgccggaggggcaaggggcacgatggcctttaccagggtctcagtacagccaccaaggacacctacgacgcccttcacatgcaggccctgccccctcgc

SEQ ID NO: 33 - DNA, 1756 bp, Artificial Sequence
  Synthesized construct
atcccacagtgcatacgtgggctccaacaggtcctcttgtcgagccacagtgcatacgtgggctccaacaggtcctcttgtcgagccacagtgcatacgtgggctccaacaggtcctcttgtcgagccacagtgcatacgtgggctccaacaggtcctcttgtcgagccacagtgcatacgtgggctccaacaggtcctcttgtcgagatctggtaggcgtgtacggtgggaggtctatataagcagagctcgtttagtgaaccgtcagatcactaggctagcatggctctgccagtgacagctctgctgctgcctctggctctgctgctgcacgcagctagacccgacatccagatgacccagagcccttcttctctgagcgccagcgtgggagacagagtgaccatcacttgcagggccagccaggacatcagcaagtacctgaattggtaccagcagaagccaggcaaggcccctagactgctgatctaccacacaagcagactgcacagcggagtgcctagcagattcagcggcagcggaagcggaaccgactacaccctgaccatcagcagcctgcagccagaggacttcgccacctactactgccagcagggcaacacactgccttacaccttcggcggaggcacaagactggagatcaagggcagcacaagcggaagcggcaaaccaggaagcggagaaggaagcaccaagggacaggtgcagctgcaggaaagcggaccaggactggtgaagccttctcagaccctgagcctgacttgcaccgtgtcaggagtgtccctgccagattacggcgtgtcttggatcagacagcccccaggaaaggccctggagtggctgggagtgatttggggaagcgagaccacctactacaacagcagcctgaagacccggctgaccatcagcaaggacaacagcaagaaccaggtggtgctgaccatgaccaacatggaccccgtggacaccgccacctactattgcgccaagcactactactacggcggaagctacgccatggactattggggccagggaagcagcgtgaccgtgtctagcctcgagaccacgacgccagcgccgcgaccaccaacaccggcgcccaccatcgcgtcgcagcccctgtccctgcgcccagaggcgtgccggccagcggcggggggcgcagtgcacacgagggggctggacttcgcctgtgatatctacatctgggcgcccttggccgggacttgtggggtccttctcctgtcactggttatcaccctttactgcaaacggggcagaaagaaactcctgtatatattcaaacaaccatttatgagaccagtacaaactactcaagaggaagatggctgtagctgccgatttccagaagaagaagaaggaggatgtgaactgagagtgaagttcagcaggagcgcagacgcccccgcgtacaagcagggccagaaccagctctataacgagctcaatctaggacgaagagaggagtacgatgttttggacaagagacgtggccgggaccctgagatggggggaaagccgagaaggaagaaccctcaggaaggcctgtacaatgaactgcagaaagataagatggcggaggcctacagtgagattgggatgaaaggcgagcgccggaggggcaaggggcacgatggcctttaccagggtctcagtacagccaccaaggacacctacgacgcccttcacatgcaggccctgccccctcgc

SEQ ID NO: 34 - DNA, 1509 bp, Artificial Sequence
  Synthesized construct
gacatccaggatatccagctgacacagtcccctagctccctgagcgcctccgtgggcgacagggtgaccatcacatgcagcgcctctagctccgtgagattcatccactggtaccagcagaagcccggcaaggcccctaagaggctgatctatgatacctctaagctggccagcggagtgccctcccgcttctctggcagcggctccggcaccgactttaccctgacaatctctagcctgcagccagaggattttgccacatactattgccagcagtggtcctctagccccttcacctttggccagggcacaaaggtggagatcaagggatctaccagcggatccggcaagcctggatctggagagggcagcacaaagggctccgaggtgcagctggtggagtccggaggaggactggtgcagccaggaggatctctgaggctgagctgtgcagcctccggcttcaacatcaaggactactatatccactgggtgagacaggcacctggcaagggactggagtgggtggcatggatcgaccctgagaatggcgataccgagttcgtgccaaagtttcagggcagggccacaatctctgccgacaccagcaagaacacagcctacctgcagatgaatagcctgcgcgccgaggataccgccgtgtactattgtaagacaggaggattttggggacagggcaccctggtgacagtgtcctctctcgaggcaccacctcgggccagcgccctgcctgcaccacccaccggctccgccctgccagaccctcagacagcatctgccctgccagatcctccagcagcaagcgccctgcccgaattcttctgggtgctggtcgtggtgggtggcgtgctggcctgctacagcctgctggtgacagtggccttcatcatcttttgggtgaggagcaagcggagcagaggcggccacagcgactacatgaacatgactccccgccgccccgggcccacccgcaagcattaccagccctatgccccaccacgcgacttcgcagcctatcgctccgttaaacggggcagaaagaaactcctgtatatattcaaacaaccatttatgagaccagtacaaactactcaagaggaagatggctgtagctgccgatttccagaagaagaagaaggaggatgtgaactgagagtgaagttcagcaggagcgcagacgcccccgcgtaccagcagggccagaaccagctctataacgagctcaatctaggacgaagagaggagtacgatgttttggacaagagacgtggccgggaccctgagatggggggaaagccgagaaggaagaaccctcaggaaggcctgtacaatgaactgcagaaagataagatggcggaggcctacagtgagattgggatgaaaggcgagcgccggaggggcaaggggcacgatggcctttaccagggtctcagtacagccaccaaggacacctacgacgcccttcacatgcaggccctgccccctcgc

SEQ ID NO: 35 - DNA, 2088 bp, Artificial Sequence
  Synthesized construct
gacatccaggatatccagctgacacagtcccctagctccctgagcgcctccgtgggcgacagggtgaccatcacatgcagcgcctctagctccgtgagattcatccactggtaccagcagaagcccggcaaggcccctaagaggctgatctatgatacctctaagctggccagcggagtgccctcccgcttctctggcagcggctccggcaccgactttaccctgacaatctctagcctgcagccagaggattttgccacatactattgccagcagtggtcctctagccccttcacctttggccagggcacaaaggtggagatcaagggatctaccagcggatccggcaagcctggatctggagagggcagcacaaagggctccgaggtgcagctggtggagtccggaggaggactggtgcagccaggaggatctctgaggctgagctgtgcagcctccggcttcaacatcaaggactactatatccactgggtgagacaggcacctggcaagggactggagtgggtggcatggatcgaccctgagaatggcgataccgagttcgtgccaaagtttcagggcagggccacaatctctgccgacaccagcaagaacacagcctacctgcagatgaatagcctgcgcgccgaggataccgccgtgtactattgtaagacaggaggattttggggacagggcaccctggtgacagtgtcctctctcgaggagagcaagtacggccctccctgccccccttgccctgcccccgagttcctgggcggacccagcgtgttcctgttcccccccaagcccaaggacaccctgatgatcagccggacccccgaggtgacctgtgtggtggtggacgtgtcccaggaggaccccgaggtccagttcaactggtacgtggacggcgtggaggtgcacaacgccaagaccaagccccgggaggagcagttcaatagcacctaccgggtggtgtccgtgctgaccgtgctgcaccaggactggctgaacggcaaggaatacaagtgtaaggtgtccaacaagggcctgcccagcagcatcgagaaaaccatcagcaaggccaagggccagcctcgggagccccaggtgtacaccctgccccctagccaagaggagatgaccaagaatcaggtgtccctgacctgcctggtgaagggcttctaccccagcgacatcgccgtggagtgggagagcaacggccagcccgagaacaactacaagaccaccccccctgtgctggacagcgacggcagcttcttcctgtacagcaggctgaccgtggacaagagccggtggcaggagggcaacgtctttagctgctccgtgatgcacgaggccctgcacaaccactacacccagaagagcctgtccctgagcctgggcaaggaattcttctgggtgctggtcgtggtgggtggcgtgctggcctgctacagcctgctggtgacagtggccttcatcatcttttgggtgaggagcaagcggagcagaggcggccacagcgactacatgaacatgactccccgccgccccgggcccacccgcaagcattaccagccctatgccccaccacgcgacttcgcagcctatcgctccgttaaacggggcagaaagaaactcctgtatatattcaaacaaccatttatgagaccagtacaaactactcaagaggaagatggctgtagctgccgatttccagaagaagaagaaggaggatgtgaactgagagtgaagttcagcaggagcgcagacgcccccgcgtaccagcagggccagaaccagctctataacgagctcaatctaggacgaagagaggagtacgatgttttggacaagagacgtggccgggaccctgagatggggggaaagccgagaaggaagaaccctcaggaaggcctgtacaatgaactgcagaaagataagatggcggaggcctacagtgagattgggatgaaaggcgagcgccggaggggcaaggggcacgatggcctttaccagggtctcagtacagccaccaaggacacctacgacgcccttcacatgcaggccctgccccctcgc

SEQ ID NO: 36 - DNA, 804 bp, Artificial Sequence
  Synthesized construct
atggccttaccagtgaccgccttgctcctgccgctggccttgctgctccacgccgccaggccggacatccagatgacccagagcccaagcagcctgagcgccagcgtgggtgacagagtgaccatcacctgtagtaccagttcgagtgtaagttacatgcactggtaccagcagaagccaggtaaggctccaaggctgctgatctacagcacatccaacctggcttctggtgtgccaagcagattcagcggtagcggtagcggtaccgacttcaccttcaccatcagcagcctccagccagaggacatcgccacctactactgccatcagtggagtagttatcccacgttcggccaagggaccaaggtggaaatcaaaggatccacttccggttcaggaaagcccgggagtggtgaaggtagcactaaaggccaggtccagctgcaggagagcggtccaggtcttgtgagacctagccagaccctgagcctgacctgcaccgtgtctggcttcaccatcagcagtggttatagctggcactgggtgagacagccacctggacgaggtcttgagtggattggatacatacagtacagtggtatcactaactacaacccctctctcaaaagtagagtgacaatgctggtagacaccagcaagaaccagttcagcctgagactcagcagcgtgacagccgccgacaccgcggtctattattgtgcaagagaagactatgattaccactggtacttcgatgtctggggtcaaggcagcacggtcaccgtctcctcaggtgcggccgcc

SEQ ID NO: 37 - DNA, 672 bp, Artificial Sequence
  Synthesized construct
accacgacgccagcgccgcgaccaccaacaccggcgcccaccatcgcgtcgcagcccctgtccctgcgcccagaggcgtgccggccagcggcggggggcgcagtgcacacgagggggctggacttcgcctgtgatatctacatctgggcgcccttggccgggacttgtggggtccttctcctgtcactggttatcaccctttactgcaaacggggcagaaagaaactcctgtatatattcaaacaaccatttatgagaccagtacaaactactcaagaggaagatggctgtagctgccgatttccagaagaagaagaaggaggatgtgaactgagagtgaagttcagcaggagcgcagacgcccccgcgtacaagcagggccagaaccagctctataacgagctcaatctaggacgaagagaggagtacgatgttttggacaagagacgtggccgggaccctgagatggggggaaagccgagaaggaagaaccctcaggaaggcctgtacaatgaactgcagaaagataagatggcggaggcctacagtgagattgggatgaaaggcgagcgccggaggggcaaggggcacgatggcctttaccagggtctcagtacagccaccaaggacacctacgacgcccttcacatgcaggccctgccccctcgctaa

SEQ ID NO: 38 - protein, 41 aa, Artificial Sequence
  Synthesized construct
RSKRSRGGHSDYMNMTPRRPGPTRKHYQPYAPPRDFAAYRS